European Patent Application EP 4 478 051 A1, published December 18, 2024. Title: 活性型オレキシンＡを定量する方法. Applicant: エーザイ・アール・アンド・ディー・マネジメント株式会社. Application JP. The sequence listing filed with the application follows.

SEQUENCE LISTING (4 sequences)

SEQ ID NO: 1 - protein, 8 aa, Homo sapiens
  MOD_RES 1: note = pyroglutamic acid
XPLPDCCR

SEQ ID NO: 2 - protein, 18 aa, Homo sapiens
  MOD_RES 18: note = amidated leucine
LYELLHGAGNHAAGILTX

SEQ ID NO: 3 - protein, 33 aa, Homo sapiens
  MOD_RES 33: note = amidated leucine
  MOD_RES 1: note = pyroglutamic acid
XPLPDCCRQKTCSCRLYELLHGAGNHAAGILTX

SEQ ID NO: 4 - protein, 5 aa, Homo sapiens
TCSCR